European Patent Specification EP 3 709 798 B1, published April 17, 2024. Title: Primate retinal pigment epithelium cell-specific promoter. Applicant: Friedrich Miescher for Biomedical Research. The sequence listing filed with the application follows.

SEQUENCE LISTING (3 sequences)

SEQ ID NO: 1 - DNA, 750 bp, Mus musculus
tcaagcctcctaccgcctttgttatgcaaacatatcaaacgccctcctttgttatgcaaaagggctggaacggggcctttgttatgcaaatcgccctccccgatccctttgttatgcaaatttgacgaattcccacctttgttatgcaaacaaatctcctaccctcctttgttatgcaaagtgagaggggctgcacctttgttatgcaaaatgcggcccctgagacctttgttatgcaaaaaccatgtacgcttgcctttgttatgcaaaccgcctgttgcttggcctttgttatgcaaagccacgcgattggcgcctttgttatgcaaagctcggttatgtacacctttgttatgcaaagctactttaaacttgcctttgttatgcaaatcacgacctgaccgtcctttgttatgcaaaaacggttgaaatagtcctttgttatgcaaaatgatattgaatagtcctttgttatgcaaaaatttagatgccgaccctttgttatgcaaaggaatgggcgtgctgcctttgttatgcaaattttcgctgcgacagcctttgttatgcaaacatgctcgccactcacctttgttatgcaaaggtctaacaatgacccctttgttatgcaaactacgtggaatagatcctttgttatgcaaaccccgagtttttgaacctttgttatgcaaaatcagtaacttcattcctttgttatgcaaaatgtgacttaacctccctttgttatgcaaa

SEQ ID NO: 2 - DNA, 214 bp, sv40
gctcgagatctgcgatctgcatctcaattagtcagcaaccatagtcccgcccctaactccgcccatcccgcccctaactccgcccagttccgcccattctccgccccatcgctgactaattttttttatttatgcagaggccgaggccgcctcggcctctgagctattccagaagtagtgaggaggcttttttggaggcctaggcttttgcaaa

SEQ ID NO: 3 - DNA, 964 bp, Mus musculus
tcaagcctcctaccgcctttgttatgcaaacatatcaaacgccctcctttgttatgcaaaagggctggaacggggcctttgttatgcaaatcgccctccccgatccctttgttatgcaaatttgacgaattcccacctttgttatgcaaacaaatctcctaccctcctttgttatgcaaagtgagaggggctgcacctttgttatgcaaaatgcggcccctgagacctttgttatgcaaaaaccatgtacgcttgcctttgttatgcaaaccgcctgttgcttggcctttgttatgcaaagccacgcgattggcgcctttgttatgcaaagctcggttatgtacacctttgttatgcaaagctactttaaacttgcctttgttatgcaaatcacgacctgaccgtcctttgttatgcaaaaacggttgaaatagtcctttgttatgcaaaatgatattgaatagtcctttgttatgcaaaaatttagatgccgaccctttgttatgcaaaggaatgggcgtgctgcctttgttatgcaaattttcgctgcgacagcctttgttatgcaaacatgctcgccactcacctttgttatgcaaaggtctaacaatgacccctttgttatgcaaactacgtggaatagatcctttgttatgcaaaccccgagtttttgaacctttgttatgcaaaatcagtaacttcattcctttgttatgcaaaatgtgacttaacctccctttgttatgcaaagctcgagatctgcgatctgcatctcaattagtcagcaaccatagtcccgcccctaactccgcccatcccgcccctaactccgcccagttccgcccattctccgccccatcgctgactaattttttttatttatgcagaggccgaggccgcctcggcctctgagctattccagaagtagtgaggaggcttttttggaggcctaggcttttgcaaa